European Patent Application EP 4 159 193 A1, published April 5, 2023. Title: MUTATED ARYLSULFATASE A. Applicant: Rheinische Friedrich-Wilhelms-Universitaet Bonn. The sequence listing filed with the application follows.

SEQUENCE LISTING (4 sequences)

SEQ ID NO: 1 - protein, 507 aa, Homo sapiens
MGAPRSLLLALAAGLAVARPPNIVLIFADDLGYGDLGCYGHPSSTTPNLDQLAAGGLRFTDFYVPVSLCTPSRAALLTGRLPVRMGMYPGVLVPSSRGGLPLEEVTVAEVLAARGYLTGMAGKWHLGVGPEGAFLPPHQGFHRFLGIPYSHDQGPCQNLTCFPPATPCDGGCDQGLVPIPLLANLSVEAQPPWLPGLEARYMAFAHDLMADAQRQDRPFFLYYASHHTHYPQFSGQSFAERSGRGPFGDSLMELDAAVGTLMTAIGDLGLLEETLVIFTADNGPETMRMSRGGCSGLLRCGKGTTYEGGVREPALAFWPGHIAPGVTHELASSLDLLPTLAALAGAPLPNVTLDGFDLSPLLLGTGKSPRQSLFFYPSYPDEVRGVFAVRTGKYKAHFFTQGSAHSDTTADPACHASSSLTAHEPPLLYDLSKDPGENYNLLGGVAGATPEVLQALKQLQLLKAQLDAAVTFGPSQVARGEDPALQICCHPGCTPRPACCHCPDPHA

SEQ ID NO: 2 - DNA, 1524 bp, Homo sapiens
  source 1..1524: mol_type = other DNA
atgggggcaccgcggtccctcctcctggccctggctgctggcctggccgttgcccgtccgcccaacatcgtgctgatctttgccgacgacctcggctatggggacctgggctgctatgggcaccccagctctaccactcccaacctggaccagctggcggcgggagggctgcggttcacagacttctacgtgcctgtgtctctgtgcacaccctctagggccgccctcctgaccggccggctcccggttcggatgggcatgtaccctggcgtcctggtgcccagctcccgggggggcctgcccctggaggaggtgaccgtggccgaagtcctggctgcccgaggctacctcacaggaatggccggcaagtggcaccttggggtggggcctgagggggccttcctgcccccccatcagggcttccatcgatttctaggcatcccgtactcccacgaccagggcccctgccagaacctgacctgcttcccgccggccactccttgcgacggtggctgtgaccagggcctggtccccatcccactgttggccaacctgtccgtggaggcgcagcccccctggctgcccggactagaggcccgctacatggctttcgcccatgacctcatggccgacgcccagcgccaggatcgccccttcttcctgtactatgcctctcaccacacccactaccctcagttcagtgggcagagctttgcagagcgttcaggccgcgggccatttggggactccctgatggagctggatgcagctgtggggaccctgatgacagccataggggacctggggctgcttgaagagacgctggtcatcttcactgcagacaatggacctgagaccatgcgtatgtcccgaggcggctgctccggtctcttgcggtgtggaaagggaacgacctacgagggcggtgtccgagagcctgccttggccttctggccaggtcatatcgctcccggcgtgacccacgagctggccagctccctggacctgctgcctaccctggcagccctggctggggccccactgcccaatgtcaccttggatggctttgacctcagccccctgctgctgggcacaggcaagagccctcggcagtctctcttcttctacccgtcctacccagacgaggtccgtggggtttttgctgtgcggactggaaagtacaaggctcacttcttcacccagggctctgcccacagtgataccactgcagaccctgcctgccacgcctccagctctctgactgctcatgagcccccgctgctctatgacctgtccaaggaccctggtgagaactacaacctgctggggggtgtggccggggccaccccagaggtgctgcaagccctgaaacagcttcagctgctcaaggcccagttagacgcagctgtgaccttcggccccagccaggtggcccggggcgaggaccccgccctgcagatctgctgtcatcctggctgcaccccccgcccagcttgctgccattgcccagatccccatgcctga

SEQ ID NO: 3 - protein, 507 aa, Homo sapiens
MGAPRSLLLALAAGLAVARPPNIVLIFADDLGYGDLGCYGHPSSTTPNLDQLAAGGLRFTDFYVPVSLCTPSRAALLTGRLPVRMGMYPGVLVPSSRGGLPLEEVTVAEVLAARGYLTGMAGKWHLGVGPEGAFLPPHQGFHRFLGIPYSHDQGPCQNLTCFPPATPCDGGCDQGLVPIPLLANLSVEAQPPWLPGLEARYVAFAHDLMADAQRQDRPFFLYYASHHTHYPQFSGQSFAERSGRGPFGDSLMELDAAVGTLMTAIGDLGLLEETLVIFTADNGPETMRMSRGGCSGLLRCGKGTTYEGGVREPALAFWPGHIAPGVTHELASSLDLLPTLAALAGAPLPNVTLDGFDLSPLLLGTGKSPRQSLFFYPSYPDEVRGVFAVRTGKYKAHFFTQGSAHSDTTADPACHASSSLTAHEPPLLYDLSKDPGENYNLLGGVAGATPEVLQALKQLQLLKAQLDAAVTFGPSQVARGEDPALQICCHPGCTPRPACCHCPDPHA

SEQ ID NO: 4 - protein, 507 aa, Homo sapiens
MGAPRSLLLALAAGLAVARPPNIVLIFADDLGYGDLGCYGHPSSTTPNLDQLAAGGLRFTDFYVPVSLCTPSRAALLTGRLPVRMGMYPGVLVPSSRGGLPLEEVTVAEVLAARGYLTGMAGKWHLGVGPEGAFLPPHQGFHRFLGIPYSHDQGPCQNLTCFPPATPCDGGCDQGLVPIPLLANLSVEAQPPWLPGLEARYVAFAHDLMADAQRQDRPFFLYYASHHTHYPQFSGQSFAERSGRGPFGDSLMELDAAVGTLMTAIGDLGLLEETLVIFTADNGPELMRMSNGGCSGLLRCGKGTTYEGGVREPALAFWPGHIAPGVTHELASSLDLLPTLAALAGAPLPNVTLDGFDLSPLLLGTGKSPRQSLFFYPSYPDEVRGVFAVRTGKYKAHFFTQGSAHSDTTADPACHASSSLTAHEPPLLYDLSKDPGENYNLLGGVAGATPEVLQALKQLQLLKAQLDAAVTFGPSQVARGEDPALQICCHPGCTPRPACCHCPDPHA